European Patent Application EP 4 741 413 A1, published May 13, 2026. Title: Novel Peptide Having Activity of Improving Dry Eye Disease and Uses Thereof. Applicant: CAREGEN CO., LTD. The sequence listing filed with the application follows.

SEQUENCE LISTING (17 sequences)

SEQ ID NO: 1 - protein, 10 aa, synthetic construct
TLKKNKRFSK

SEQ ID NO: 2 - DNA, 20 bp, synthetic construct
  source 1..20: mol_type = other DNA
cgactactacaaccctccgc

SEQ ID NO: 3 - DNA, 20 bp, synthetic construct
  source 1..20: mol_type = other DNA
gggaggagttggtacacacg

SEQ ID NO: 4 - DNA, 20 bp, synthetic construct
  source 1..20: mol_type = other DNA
aaggtggctgaccaagatgg

SEQ ID NO: 5 - DNA, 20 bp, synthetic construct
  source 1..20: mol_type = other DNA
tctcgtttgtcatcaccccg

SEQ ID NO: 6 - DNA, 21 bp, synthetic construct
  source 1..21: mol_type = other DNA
atcattcaccaggcaaattgc

SEQ ID NO: 7 - DNA, 21 bp, synthetic construct
  source 1..21: mol_type = other DNA
ggcttcagcataaagcgtttg

SEQ ID NO: 8 - DNA, 20 bp, synthetic construct
  source 1..20: mol_type = other DNA
ttcgacacatgggataacga

SEQ ID NO: 9 - DNA, 20 bp, synthetic construct
  source 1..20: mol_type = other DNA
tctttcaacacgcaggacag

SEQ ID NO: 10 - DNA, 20 bp, synthetic construct
  source 1..20: mol_type = other DNA
aaagaggcactgccagaaaa

SEQ ID NO: 11 - DNA, 20 bp, synthetic construct
  source 1..20: mol_type = other DNA
atctgaggtgcccatgctac

SEQ ID NO: 12 - DNA, 27 bp, synthetic construct
  source 1..27: mol_type = other DNA
caaaacatatttctttgtagaggacaa

SEQ ID NO: 13 - DNA, 20 bp, synthetic construct
  source 1..20: mol_type = other DNA
ttcagctatttgcttgggaa

SEQ ID NO: 14 - DNA, 20 bp, synthetic construct
  source 1..20: mol_type = other DNA
gggacgcagacatcgtcatc

SEQ ID NO: 15 - DNA, 20 bp, synthetic construct
  source 1..20: mol_type = other DNA
tcgtcatcgtcgaaatgggc

SEQ ID NO: 16 - DNA, 20 bp, synthetic construct
  source 1..20: mol_type = other DNA
ggagccaaaagggtcatcat

SEQ ID NO: 17 - DNA, 20 bp, synthetic construct
  source 1..20: mol_type = other DNA
gtgatggcatggactgtggt